European Patent Application EP 4 591 867 A2, published July 30, 2025. Title: Methods for detecting Bordetella. Applicant: Quest Diagnostics Investments LLC. Application EP EP22189467.8, filed August 9, 2022. The sequence listing filed with the application follows.

SEQUENCE LISTING (20 sequences)

SEQ ID NO: 1 - DNA, 85 bp, Bordetella pertussis
  source 1..85: mol_type = other DNA
ccataagcatgcccgattgaccttcctacgtcgactcgaaatggtccagcaattgatcgcccatcaagtttgtgtgcctgaagcg

SEQ ID NO: 2 - DNA, 65 bp, Bordetella parapertussis
  source 1..65: mol_type = other DNA
cggctcgacgaattgctgcaagccaaccagccgctgctgacggtctatgtcctgcgtgacgaact

SEQ ID NO: 3 - DNA, 133 bp, Bordetella holmesii
  source 1..133: mol_type = other DNA
ggcacggatcgaggtttttgcgattgcgcagcagtagccagcgactggacttgatcacccggcgggccggcttgtcgtgccgcaactggttcgcttggtctacacgcacccggtctatcacttcacggccgta

SEQ ID NO: 4 - DNA, 19 bp, synthetic construct
  misc_feature 1..19: note = Description of Artificial Sequence: Syntheticprimer
  source 1..19: mol_type = other DNA
ggcacggatcgaggttttt

SEQ ID NO: 5 - DNA, 20 bp, synthetic construct
  misc_feature 1..20: note = Description of Artificial Sequence: Syntheticprimer
  source 1..20: mol_type = other DNA
tacggccgtgaagtgataga

SEQ ID NO: 6 - DNA, 22 bp, synthetic construct
  misc_feature 1..22: note = Description of Artificial Sequence: Syntheticprobe
  source 1..22: mol_type = other DNA
agtcgctggctactgctgcgca

SEQ ID NO: 7 - DNA, 16 bp, synthetic construct
  misc_feature 1..16: note = Description of Artificial Sequence: Syntheticprimer
  source 1..16: mol_type = other DNA
cggctcgacgaattgc

SEQ ID NO: 8 - DNA, 19 bp, synthetic construct
  misc_feature 1..19: note = Description of Artificial Sequence: Syntheticprimer
  source 1..19: mol_type = other DNA
agttcgtcacgcaggacat

SEQ ID NO: 9 - DNA, 22 bp, synthetic construct
  misc_feature 1..22: note = Description of Artificial Sequence: Syntheticprobe
  source 1..22: mol_type = other DNA
caaccagccgctgctgacggtc

SEQ ID NO: 10 - DNA, 19 bp, synthetic construct
  misc_feature 1..19: note = Description of Artificial Sequence: Syntheticprimer
  source 1..19: mol_type = other DNA
cgcttcaggcacacaaact

SEQ ID NO: 11 - DNA, 18 bp, synthetic construct
  misc_feature 1..18: note = Description of Artificial Sequence: Syntheticprimer
  source 1..18: mol_type = other DNA
ccataagcatgcccgatt

SEQ ID NO: 12 - DNA, 27 bp, synthetic construct
  misc_feature 1..27: note = Description of Artificial Sequence: Syntheticprobe
  source 1..27: mol_type = other DNA
tcaattgctggaccatttcgagtcgac

SEQ ID NO: 13 - DNA, 577 bp, synthetic construct
  misc_feature 1..577: note = Description of Artificial Sequence: Syntheticpolynucleotide
  source 1..577: mol_type = other DNA
taaccccgcgataaagacagaagattatgcatacgagatcaaaggagccggccttttctctagagatctcttattttccttgaagtcacctgtttatgttaaagcaggtgagcaggtatacattcagtacgatctgaacaaaagcaatgcagaacttgctctcgactatggttttgtggaatcaaaccctaaacggaactcatatactttaacaatagagataccagaatcagacccattctttggggataagttggatattgctgagagtaacaagatgggtgagaccggatactttgacatagtagacggccagactcttcccgctggtatgcttcagtaccttcggcttgtggctcttggcggtccagatgctttcttattagaatctatcttcaataacaccatatggggtcatcttgaattgcctgtaagtcgtacaaacgaggaactcatatgccgtgttgtcagagatgcctgcaaatctgctctgtctggttttgatacgaccattgaagaggatgagaagcttctggacaaaggaaagcttgagcctaggttggaaatggctctcaag

SEQ ID NO: 14 - DNA, 446 bp, Bordetella holmesii
  source 1..446: mol_type = other DNA
gtgttgtyaatgccctcaacgatgctggtgttgagccggtggcgacagcgagacagaatcccgtgcagataggcttttagcttgagcgcgaagtgagccaaggcggcgatgccgctgccctgagcctgttgcagccagtgatcccatgcctggcgggcgtagccggggtgttggtagaaccacagctgtttgagctcatcgcgcatcagataagcggtgagcaagggctggttggcctggagcaactcgtccaactttaccgattggcacggatcgaggtttttgcgattgcgcagcagtagccagcgactggacttgatcacccggcgggccggcttgtcgtgccgcaactggttcgcttggtctacacgcacccggtctatcacttcacggccgtacttggccacgacgtggaacaggtcgtagacgatctcggcgttggggca

SEQ ID NO: 15 - DNA, 1190 bp, Bordetella parapertussis
  source 1..1190: mol_type = other DNA
gctggatcgcaagttgatggagtcgctgggaggctggcagggctatggcgtcgaacgcgtggaatggcccgaagacccagggcgcacgctgtcgatctatttgaagccaacggccaaggtgatgctgtgcgagcagtgcggcgcgcggtgtcgccaggtgcatgagaccacggttcgacgggtgcgagatctgccgttattcgagtatcgggtcgttctgcacgtgccgcgccgacgcttgtggtgtgagcaatgcggcggcccgcgcctggagcggcttgcctggctggggcgatatcaacgggtgacggatcggctggcgcaggcctgcagccaattgctgcaatcgagcaacgtgcaggcggtggcgaggttcttcgagctgggttggcataccgtcaagacgctggacaaggctcggctgcgtgcgtcggtgcgcgaaccggattggtccaagatcgagtatttggcgatggacgagtttgccctgcacaaagggcatcgctacgcgacagtggtggtcgatccgatcggcaggcaggtgctgtggattggcccaggacgctcacgcgagacggcccgggcgttcttcgaacaattgccgcctggggccgcccaacgcatcaaggccgttgccatcgacatgaccaccgcctacgagttggagatccaggcccacagcccacaggcggagatcgtctatgacttgttccatgtcgtggccaagtatggacgagaggtcattgatcgggtgcgcgtggatcaggccaatcaactacgccaggatcgtcccgcacgcaggatcatcaaatcgagtcgctggctgctgctgcgcaaccgtgacaacctggatcggcagcaggccgtccggctcgacgaattgctgcaagccaaccagccgctgctgacggtctatgtcctgcgtgacgaactcaaacggctctggttctaccaaagacctgcctgggcaagacaagcctggaaccactggtacgagcaggccgagcaaagcggaatagccgccttgaacaccttcgctcagcgcttgaaaggctatctgcacggcatcctggccagatgccgacatcccctgaacaccagcattgtcgagggcatcaacaacactatcaaggtcatcaagcggcgcgcttacggctaccgcgaccaggaatacttcttcctcaaaatcc

SEQ ID NO: 16 - DNA, 1055 bp, Bordetella pertussis
  source 1..1055: mol_type = other DNA
gttaggtgtgaagattcaataggttgtatgcatggttcatccgaaccggatttgagaaactggaaatcgccacccccccagttcactcaaggagcccggccggatgaacacccataagcatgcccgattgaccttcctacgtcgactcgaaatggtccagcaattgatcgcccatcaagtttgtgtgcctgaagcggcccgcgcctatggggtcaccgcgccgactgtgcgcaaatggctgggccgcttcctggctcagggccaggcgggcttggccgatgcgtcctcgcgcccgacggtctcgccccgagcgattgcgccggccaaggcgctggctatcgtggagctgcgccgcaagcggctgacccaagcgcgcatcgcccaggcgctgggcgtgtcagccagcaccgtcagccgcgtcctggcccgcgccggtctgtcgcacctggccgacctggagccggccgagccggtggtgcgctacgagcatcaggcccccggcgatctgctgcacatcgacatcaagaagctgggacgtatccagcgccctggccaccgggtcacgggccaccgacgcgataccgttgagggggccggctgggacttcgtcttcgtggccatcgatgaccacgcccgcgtggccttcaccgacatccaccccgacgagcgcttccccagcgccgtccagttcctcaaggacgcagtggcctactaccagcgcctgggcgtgaccatccagcgcttgctcaccgacaatggctcggcctttcgcagccgcgccttcgccgcgctgtgccatgagctgggcatcaagcaccgctttacccgaccttaccgcccacagaccaatggcaaggccgaacgcttcatccagtcggccttgcgtgagtgggcttacgctcacacctaccagaactcccaacaccgagccgatgccatgaaatcctggttacaccactacaactggcatcgaccccaccaaggcatcgggcgcgctgtacccatctccagactcaacctggacgaatacaacctattgacagttcacagttagg

SEQ ID NO: 17 - DNA, 20 bp, synthetic construct
  misc_feature 1..20: note = Description of Artificial Sequence: Syntheticprimer
  source 1..20: mol_type = other DNA
gcttcagtaccttcggcttg

SEQ ID NO: 18 - DNA, 20 bp, synthetic construct
  misc_feature 1..20: note = Description of Artificial Sequence: Syntheticprimer
  source 1..20: mol_type = other DNA
ttgcaggcatctctgacaac

SEQ ID NO: 19 - DNA, 21 bp, synthetic construct
  misc_feature 1..21: note = Description of Artificial Sequence: Syntheticprobe
  source 1..21: mol_type = other DNA
tggctcttggcggtccagatg

SEQ ID NO: 20 - DNA, 150 bp, synthetic construct
  misc_feature 1..150: note = Description of Artificial Sequence: Syntheticpolynucleotide
  source 1..150: mol_type = other DNA
gcttcagtaccttcggcttgtggctcttggcggtccagatgctttcttattagaatctatcttcaataacaccatatggggtcatcttgaattgcctgtaagtcgtacaaacgaggaactcatatgccgtgttgtcagagatgcctgcaa